European Patent Application EP 4 276 192 A1, published November 15, 2023. Title: Analytical method and therapeutical agent for use in combination with L-asparaginase in tumour therapy. Applicant: Medizinische Hochschule Hannover. The sequence listing filed with the application follows.

SEQUENCE LISTING (4 sequences)

SEQ ID NO: 1 - DNA, 21 bp, Artificial Sequence
  shRNA TRCN0000005942
ataaggcctgttgttccttgc

SEQ ID NO: 2 - DNA, 21 bp, Artificial Sequence
  TRCN0000005939
aaagagcttaacatactcagc

SEQ ID NO: 3 - DNA, 20 bp, Artificial Sequence
  sgUBR2 #3
gaaacttgaaatagtctaaa

SEQ ID NO: 4 - DNA, 20 bp, Artificial Sequence
  sgAAVS1
agcggctccaattcggaagt